European Patent Specification EP 3 262 077 B1, published June 4, 2025. Title: Acinetobacter O-Oligosaccharyltransferases and Uses Thereof. Applicant: VaxAlta Inc. The sequence listing filed with the application follows.

SEQUENCE LISTING (90 sequences)

SEQ ID NO: 1 - DNA, 28 bp, Artificial Sequence
  primer
agaatacttgcatagtgacaggttacag

SEQ ID NO: 2 - DNA, 21 bp, Artificial Sequence
  primer
gttatggcggcggtggaggtc

SEQ ID NO: 3 - DNA, 70 bp, Artificial Sequence
  primer
caaaaagcttatataaaaacatacatacaatctttggggaaaaggctatgattccggggatccgtcgacc

SEQ ID NO: 4 - DNA, 70 bp, Artificial Sequence
  primer
ggattgacctctcttttttatttctaaaattacgatgctacaaatgattgtgtaggctggagctgcttcg

SEQ ID NO: 5 - DNA, 33 bp, Artificial Sequence
  primer
gcgggatccgcaaattggtgatgtgatgtctcg

SEQ ID NO: 6 - DNA, 33 bp, Artificial Sequence
  primer
gcgggtaccgctgcgaggaataaaaagaatact

SEQ ID NO: 7 - DNA, 33 bp, Artificial Sequence; identical to SEQ ID NO: 5
  primer

SEQ ID NO: 8 - DNA, 33 bp, Artificial Sequence
  primer
gcgggtacctcgtattgtgaactagaccatcct

SEQ ID NO: 9 - DNA, 33 bp, Artificial Sequence; identical to SEQ ID NO: 5
  primer

SEQ ID NO: 10 - DNA, 33 bp, Artificial Sequence; identical to SEQ ID NO: 6
  primer

SEQ ID NO: 11 - DNA, 28 bp, Artificial Sequence
  primer
agaatacttgcatagtgacaggttacag

SEQ ID NO: 12 - DNA, 24 bp, Artificial Sequence
  primer
cgcatttatatttggggattactc

SEQ ID NO: 13 - DNA, 70 bp, Artificial Sequence
  primer
cttccatgtataattcttctcaagtttttggtctgtaacctgtcactatgattccggggatccgtcgacc

SEQ ID NO: 14 - DNA, 70 bp, Artificial Sequence
  primer
aaaatccccttgaaaacaaggggatttttttatttatcttttaataattgtgtaggctggagctgcttcg

SEQ ID NO: 15 - DNA, 44 bp, Artificial Sequence
  primer
cttcctcaatcatttgtagcagcgtaattttagaaataaaaaag

SEQ ID NO: 16 - DNA, 44 bp, Artificial Sequence
  primer
cttttttatttctaaaattacgctgctacaaatgattgaggaag

SEQ ID NO: 17 - DNA, 23 bp, Artificial Sequence
  primer
atgaaaaaacttgagcaccttgc

SEQ ID NO: 18 - DNA, 21 bp, Artificial Sequence
  primer
tgtttgctcttatttctactg

SEQ ID NO: 19 - DNA, 23 bp, Artificial Sequence
  primer
ttgtcatttataaagttagtcac

SEQ ID NO: 20 - DNA, 24 bp, Artificial Sequence
  primer
tgtacacctgattttaatattcta

SEQ ID NO: 21 - DNA, 36 bp, Artificial Sequence
  primer
gaaataagagcaaacaattccggggatccgtcgacc

SEQ ID NO: 22 - DNA, 35 bp, Artificial Sequence
  primer
ctttataaatgacaatgtaggctggagctgcttcg

SEQ ID NO: 23 - DNA, 37 bp, Artificial Sequence
  primer set 12F
ctcaagttttttcatcgccatggcggccgggagcatg

SEQ ID NO: 24 - DNA, 40 bp, Artificial Sequence
  primer set 12R
aaaatcaggtgtacaactagtgaattcgcggccgcctgca

SEQ ID NO: 25 - DNA, 18 bp, Artificial Sequence
  primer set 13F
cgtccccaaaagcgtgaa

SEQ ID NO: 26 - DNA, 23 bp, Artificial Sequence
  primer set 13R
ttaggcaaatttcgaagcgtgat

SEQ ID NO: 27 - DNA, 28 bp, Artificial Sequence
  primer set 14F
gcgcccgggataagtgctcaattgatgg

SEQ ID NO: 28 - DNA, 25 bp, Artificial Sequence
  primer set 14R
ggtaccgagatcccaaaccagcaac

SEQ ID NO: 29 - DNA, 25 bp, Artificial Sequence
  primer set 15F
actagtgaattcgcggccgcctgca

SEQ ID NO: 30 - DNA, 22 bp, Artificial Sequence
  primer set 15R
cgccatggcggccgggagcatg

SEQ ID NO: 31 - DNA, 20 bp, Artificial Sequence
  primer set 16F
attccggggatccgtcgacc

SEQ ID NO: 32 - DNA, 20 bp, Artificial Sequence
  primer set 16R
tgtaggctggagctgcttcg

SEQ ID NO: 33 - DNA, 38 bp, Artificial Sequence
  primer set 17F
ccggccgccatggcgatgacgattggtttaattttttc

SEQ ID NO: 34 - DNA, 40 bp, Artificial Sequence
  primer set 17R
acggatccccggaatcatacttgtaaaaaaaaaagtattt

SEQ ID NO: 35 - DNA, 40 bp, Artificial Sequence
  primer set 18F
cagctccagcctacaatggaagaaaattctttattaattt

SEQ ID NO: 36 - DNA, 37 bp, Artificial Sequence
  primer set 18R
cgcgaattcactagtttaaacatatttttcccatttc

SEQ ID NO: 37 - DNA, 32 bp, Artificial Sequence
  primer set 19F
ccggccgccatggcgatgactcctgccggagg

SEQ ID NO: 38 - DNA, 41 bp, Artificial Sequence
  primer set 19R
acggatccccggaatttaataaagaattttcttccatttac

SEQ ID NO: 39 - DNA, 41 bp, Artificial Sequence
  primer set 20F
cagctccagcctacaatagtaggactaaaaaaatgatttcg

SEQ ID NO: 40 - DNA, 40 bp, Artificial Sequence
  primer set 20R
cgcgaattcactagtttatttatataaccctttttctttc

SEQ ID NO: 41 - DNA, 40 bp, Artificial Sequence
  primer set 21F
cggccgccatggcgatgtttaaaaatgtattaattactgg

SEQ ID NO: 42 - DNA, 40 bp, Artificial Sequence
  primer set 21R
acggatccccggaatcatttatttatataaccctttttct

SEQ ID NO: 43 - DNA, 40 bp, Artificial Sequence
  primer set 22F
cagctccagcctacaataaatttaaaatattcataaatct

SEQ ID NO: 44 - DNA, 40 bp, Artificial Sequence
  primer set 22R
cgcgaattcactagtttataatttaagttcttgaatcaac

SEQ ID NO: 45 - DNA, 24 bp, Artificial Sequence
  primer set 23F
ctacattgtttatttttaccagaa

SEQ ID NO: 46 - DNA, 22 bp, Artificial Sequence
  primer set 23R
gaagcttgaagttatccacgaa

SEQ ID NO: 47 - DNA, 26 bp, Artificial Sequence
  primer set 24F
catcaaaaataccagcctaaattatc

SEQ ID NO: 48 - DNA, 23 bp, Artificial Sequence
  primer set 24R
ccattgtttgaaattatttaggg

SEQ ID NO: 49 - DNA, 26 bp, Artificial Sequence
  primer set 25F
catcaaaaataccagcctaaattatc

SEQ ID NO: 50 - DNA, 25 bp, Artificial Sequence
  primer set 25R
gaagaaaattctttattaatttctg

SEQ ID NO: 51 - DNA, 26 bp, Artificial Sequence
  primer set 26F
catcaaaaataccagcctaaattatc

SEQ ID NO: 52 - DNA, 24 bp, Artificial Sequence
  primer set 26R
gaaaaagggttatataaataaatg

SEQ ID NO: 53 - DNA, 33 bp, Artificial Sequence
  primer set 27F
gcgcccgggctacattgtttatttttaccagaa

SEQ ID NO: 54 - DNA, 33 bp, Artificial Sequence
  primer set 27R
gcgggtaccaccatcattgactactaagacctc

SEQ ID NO: 55 - DNA, 33 bp, Artificial Sequence; identical to SEQ ID NO: 53
  primer set 28F

SEQ ID NO: 56 - DNA, 31 bp, Artificial Sequence
  primer set 28R
gcgggtaccttctacatccaataccagtcgt

SEQ ID NO: 57 - DNA, 33 bp, Artificial Sequence; identical to SEQ ID NO: 53
  primer set 29F

SEQ ID NO: 58 - DNA, 31 bp, Artificial Sequence
  primer set 29R
gcgggtaccgaagcttgaagttatccacgaa

SEQ ID NO: 59 - DNA, 31 bp, Artificial Sequence
  primer set 30F
gcgcccgggccgaagcagggtgggtgttagt

SEQ ID NO: 60 - DNA, 50 bp, Artificial Sequence
  primer set 30R
gcgggtaccttagtggtggtggtggtgttgagctactgaaaactcaatac

SEQ ID NO: 61 - DNA, 36 bp, Artificial Sequence
  primer set 31F
gccatatggcttatcaaaactatattgctaaatctc

SEQ ID NO: 62 - DNA, 37 bp, Artificial Sequence
  primer set 31R
gcggatccctcttttttatttctaaaattacgatgct

SEQ ID NO: 63 - DNA, 33 bp, Artificial Sequence
  primer set 32F
ataggatccatgaatgcacaaaagggttttacc

SEQ ID NO: 64 - DNA, 48 bp, Artificial Sequence
  primer set 32R
tatgtcgactcagtggtggtggtggtggtgaccacgacattctgatgg

SEQ ID NO: 65 - DNA, 34 bp, Artificial Sequence
  primer set 33F
atatggatccgtggttgatagtagtactatatgg

SEQ ID NO: 66 - DNA, 61 bp, Artificial Sequence
  primer set 33R
atatgtcgactcagtggtggtggtggtggtgatattctattgaacaaaattttaacttagg

SEQ ID NO: 67 - DNA, 40 bp, Artificial Sequence
  primer set 34F
atatggatccgtggctggttccccgcgtgtgtataatagc

SEQ ID NO: 68 - DNA, 55 bp, Artificial Sequence
  primer set 34R
atatgtcgacttagtggtggtggtggtggtgcttggatgactctacagcagaagc

SEQ ID NO: 69 - DNA, 35 bp, Artificial Sequence
  primer set 35F
actgggatccatgttaaaaaaaattattctatttc

SEQ ID NO: 70 - DNA, 64 bp, Artificial Sequence
  primer set 35R
actggtcgactaagtggtggtggtggtggtggtggtggtggtgaggaatttttgaggttggtac

SEQ ID NO: 71 - DNA, 31 bp, Artificial Sequence
  primer set 36F
actgggatccatgcaagtattctttctgttc

SEQ ID NO: 72 - DNA, 65 bp, Artificial Sequence
  primer set 36R
actggtcgactaagtggtggtggtggtggtggtggtggtggtgtttattttttaacaactctgcc

SEQ ID NO: 73 - DNA, 16 bp, Artificial Sequence
  primer set 37F
ggtggacgtggaggag

SEQ ID NO: 74 - DNA, 23 bp, Artificial Sequence
  primer set 37R
cttgcttgggttacatcagtgct

SEQ ID NO: 75 - DNA, 20 bp, Artificial Sequence
  primer set 38F
aattattgtacagccttttg

SEQ ID NO: 76 - DNA, 45 bp, Artificial Sequence
  primer set 38R
catcatcatcatcatcactaatattaaaaatgtataaaaaacacc

SEQ ID NO: 77 - DNA, 40 bp, Artificial Sequence
  primer set 39F
ccagttgaattacttcctcaagcatttgtagcatcgtaat

SEQ ID NO: 78 - DNA, 40 bp, Artificial Sequence
  primer set 39R
attacgatgctacaaatgcttgaggaagtaattcaactgg

SEQ ID NO: 79 - protein, 27 aa, Acinetobacter baylyi
SSELEDLFNSDGGAASEPAASDKTAAK

SEQ ID NO: 80 - protein, 26 aa, Acinetobacter baylyi
KLAEPAASAVADQNSPLSAQQQLEQK

SEQ ID NO: 81 - protein, 24 aa, Acinetobacter baylyi
IDAAADHAAASTEHAADKAEVATR

SEQ ID NO: 82 - protein, 26 aa, Acinetobacter baylyi
SASKPNVEASVSSQNATLSASQPQHQ

SEQ ID NO: 83 - protein, 11 aa, Acinetobacter baylyi
AAHAASAAASK

SEQ ID NO: 84 - protein, 12 aa, Acinetobacter baylyi
DAAHDAAASVEK

SEQ ID NO: 85 - protein, 18 aa, Acinetobacter baylyi
IDAAADHAAASTEHAADK

SEQ ID NO: 86 - protein, 34 aa, Acinetobacter baylyi
IYQNTDTSSAASQTSASPTTQGLGDFLHAQEQLR

SEQ ID NO: 87 - protein, 13 aa, Acinetobacter baylyi
NTAASSVAATHKK

SEQ ID NO: 88 - protein, 26 aa, Acinetobacter baylyi
VEQIVAQPAPASSVQFKPSNPEIDYK

SEQ ID NO: 89 - DNA, 33 bp, Artificial Sequence
  primer igrF
actggtcgactagtagtactatatggctttaaa

SEQ ID NO: 90 - DNA, 38 bp, Artificial Sequence
  primer igrR
actgctgcagttaatattctattgaacaaaattttaac